European Patent Specification EP 3 646 876 B1, published February 14, 2024. Title: USE OF TELOMERASE INHIBITORS FOR THE TREATMENT OF MYELOPROLIFERATIVE DISORDERS AND MYELOPROLIFERATIVE NEOPLASMS. Applicant: Stuart, Monic J Kelsey, Stephen. Application PCT/US2013/070437. The sequence listing filed with the application follows.

SEQUENCE LISTING (23 sequences)

SEQ ID NO: 1 - RNA, 554 nt, Homo sapiens
ggguugcggagggugggccugggaggggugguggccauuuuuugucuaacccuaacugagaagggcguaggcgccgugcuuuugcuccccgcgcgcuguuuuucucgcugacuuucagcgggcggaaaagccucggccugccgccuuccaccguucauucuagagcaaacaaaaaaugucagcugcuggcccguucgccucccggggaccugcggcgggucgccugcccagcccccgaaccccgccuggagccgcggucggcccggggcuucuccggaggcacccacugccaccgcgaagaguugggcucugucagccgcgggucucucgggggcgagggcgagguucaccguuucaggccgcaggaagaggaacggagcgagucccgccgcggcgcgauucccugagcugugggacgugcacccaggacucggcucacacaugcaguucgcuuuccuguugguggggggaacgccgaucgugcgcauccgucaccccucgccggcagugggggcuugugaacccccaaaccugacugacugggccagugugcu

SEQ ID NO: 2 - DNA, 20 bp, Homo sapiens
acattttttgtttgctctag

SEQ ID NO: 3 - DNA, 30 bp, Homo sapiens
gctctagaatgaacggtggaaggcggcagg

SEQ ID NO: 4 - DNA, 14 bp, Homo sapiens
gtggaggcggcagg

SEQ ID NO: 5 - DNA, 13 bp, Homo sapiens
ggaaggcggcagg

SEQ ID NO: 6 - DNA, 13 bp, Homo sapiens
gtggaaggcggca

SEQ ID NO: 7 - DNA, 11 bp, Homo sapiens
gtggaaggcgg

SEQ ID NO: 8 - DNA, 13 bp, Homo sapiens
cggtggaaggcgg

SEQ ID NO: 9 - DNA, 13 bp, Homo sapiens
acggtggaaggcg

SEQ ID NO: 10 - DNA, 16 bp, Homo sapiens
aacggtggaaggcggc

SEQ ID NO: 11 - DNA, 18 bp, Homo sapiens
atgaacggtggaaggcgg

SEQ ID NO: 12 - DNA, 13 bp, Homo sapiens
tagggttagacaa

SEQ ID NO: 13 - DNA, 13 bp, Homo sapiens
cagttagggttag

SEQ ID NO: 14 - DNA, 12 bp, Homo sapiens
tagggttagaca

SEQ ID NO: 15 - DNA, 11 bp, Homo sapiens
tagggttagac

SEQ ID NO: 16 - DNA, 11 bp, Homo sapiens
gttagggttag

SEQ ID NO: 17 - DNA, 13 bp, Homo sapiens
gttagggttagac

SEQ ID NO: 18 - DNA, 15 bp, Homo sapiens
gttagggttagacaa

SEQ ID NO: 19 - DNA, 9 bp, Homo sapiens
gggttagac

SEQ ID NO: 20 - DNA, 9 bp, Homo sapiens
cagttaggg

SEQ ID NO: 21 - DNA, 12 bp, Homo sapiens
cccttctcagtt

SEQ ID NO: 22 - DNA, 12 bp, Homo sapiens
cgcccttctcag

SEQ ID NO: 23 - RNA, 11 nt, Artificial sequence
  hTR template inhibitor
cuaacccuaac